European Patent Specification EP 3 736 572 B1, published July 24, 2024. Title: Intra-droplet surface engineering to capture a molecular target. Applicant: Université de Strasbourg Centre International de Recherche aux Frontières de la Chimie Centre National de la Recherche Scientifique. The sequence listing filed with the application follows.

SEQUENCE LISTING (13 sequences)

SEQ ID NO: 1 - DNA, 35 bp, Artificial Sequence
  Amino-modified oligonucleotide
  misc_feature (1)..(1): 5' Amino Modifier C12 and Internal Cy5TM
gatacgaattcgggtgttctgctggtagtggtcgg

SEQ ID NO: 2 - DNA, 34 bp, Artificial Sequence
  Complementary oligonucleotide
  misc_feature (1)..(1): 5'Atto(TM) 488 (NHS ester)
  misc_feature (1)..(1): 5'Atto 488 (NHS ester)
ccactaccagcagaacacccccagaattcgtatc

SEQ ID NO: 3 - DNA, 18 bp, Artificial Sequence
  amino-modified oligonucleotide
  misc_feature (1)..(1): 5' Amino Modifier C12
  misc_feature (18)..(18): 3' Cy5 introduced on supported resin
ttgctgtagccaaattcg

SEQ ID NO: 4 - DNA, 18 bp, Artificial Sequence
  Complementary oligonucleotide
  misc_feature (18)..(18): 3' Atto 488 (NHS ester).
cgaatttggctacagcaa

SEQ ID NO: 5 - DNA, 18 bp, Artificial Sequence
  amino modified oligonucleotide
  misc_feature (1)..(1): 5' Amino Modifier C12
  misc_feature (18)..(18): 3' Cy5 introduced on supported resin
ttgctgtagccaaattcg

SEQ ID NO: 6 - DNA, 18 bp, Artificial Sequence
  Complementary oligonucleotide
  misc_feature (18)..(18): 3' Atto 488 (NHS ester)
cgaatttggctacagcaa

SEQ ID NO: 7 - DNA, 27 bp, Artificial Sequence
  Amino modified oligonucleotide
  misc_feature (1)..(1): 5' Amino Modifier C12
ttgcagttttttttttttttttttttt

SEQ ID NO: 8 - DNA, 27 bp, Artificial Sequence
  Complementary oligonucleotide
  misc_feature (1)..(1): 5' Atto 488 (NHS ester)
ttgatccaaaaaaaaaaaaaaaaaaaa

SEQ ID NO: 9 - DNA, 987 bp, Artificial Sequence
  Template GAPDH DNA
taatacgactcactatagggatggggaaggtgaaggtcggagtcaacggatttggtcgtattgggcgcctggtcaccagggctgcttttaactctggtaaagtggatattgttgccatcaatgaccccttcattgacctcaactacatggtttacatgttccaatatgattccacccatggcaaattccatggcaccgtcaaggctgagaacgggaagcttgtcatcaatggaaatcccatcaccatcttccaggagcgagatccctccaaaatcaagtggggcgatgctggcgctgagtacgtcgtggagtccactggcgtcttcaccaccatggagaaggctggggctcatttgcaggggggagccaaaagggtcatcatctctgccccctctgctgatgcccccatgttcgtcatgggtgtgaaccatgagaagtatgacaacagcctcaagatcatcagcaatgcctcctgcaccaccaactgcttagcacccctggccaaggtcatccatgacaactttggtatcgtggaaggactcatgaccacagtccatgccatcactgccacccagaagactgtggatggcccctccgggaaactgtggcgtgatggccgcggggctctccagaacatcatccctgcctctactggcgctgccaaggctgtgggcaaggtcatccctgagctgaacgggaagctcactggcatggccttccgtgtccccactgccaacgtgtcagtggtggacctgacctgccgtctagaaaaacctgccaaatatgatgacatcaagaaggtggtgaagcaggcgtcggagggccccctcaagggcatcctgggctacactgagcaccaggtggtctcctctgacttcaacagcgacacccactcctccacctttgacgctggggctggcattgccctcaacgaccactttgtcaagctcatttcctggtatgacaacgaatttggctacagcaaca

SEQ ID NO: 10 - DNA, 53 bp, Artificial Sequence
  GAPDH forward primer
ggaacttgaattctaatacgactcactatagggatggggaaggtgaaggtcgg

SEQ ID NO: 11 - DNA, 20 bp, Artificial Sequence
  GAPDH reverse primer
tgttgctgtagccaaattcg

SEQ ID NO: 12 - RNA, 970 nt, Artificial Sequence
  GAPDH RNA fragment
gggauggggaaggugaaggucggagucaacggauuuggucguauugggcgccuggucaccagggcugcuuuuaacucugguaaaguggauauuguugccaucaaugaccccuucauugaccucaacuacaugguuuacauguuccaauaugauuccacccauggcaaauuccauggcaccgucaaggcugagaacgggaagcuugucaucaauggaaaucccaucaccaucuuccaggagcgagaucccuccaaaaucaaguggggcgaugcuggcgcugaguacgucguggaguccacuggcgucuucaccaccauggagaaggcuggggcucauuugcaggggggagccaaaagggucaucaucucugcccccucugcugaugcccccauguucgucaugggugugaaccaugagaaguaugacaacagccucaagaucaucagcaaugccuccugcaccaccaacugcuuagcaccccuggccaaggucauccaugacaacuuugguaucguggaaggacucaugaccacaguccaugccaucacugccacccagaagacuguggauggccccuccgggaaacuguggcgugauggccgcggggcucuccagaacaucaucccugccucuacuggcgcugccaaggcugugggcaaggucaucccugagcugaacgggaagcucacuggcauggccuuccguguccccacugccaacgugucagugguggaccugaccugccgucuagaaaaaccugccaaauaugaugacaucaagaagguggugaagcaggcgucggagggcccccucaagggcauccugggcuacacugagcaccagguggucuccucugacuucaacagcgacacccacuccuccaccuuugacgcuggggcuggcauugcccucaacgaccacuuugucaagcucauuuccugguaugacaacgaauuuggcuacagcaaca

SEQ ID NO: 13 - DNA, 18 bp, Artificial Sequence
  Capture DNA
  misc_feature (1)..(1): 5'-NH2-C12
ttgctgtagccaaattcg